European Patent Specification EP 3 653 225 B1, published October 2, 2024. Title: METHODS FOR TREATING OR PREVENTING MIGRAINE HEADACHE. Applicant: AMGEN INC. Application EP. The sequence listing filed with the application follows.

SEQUENCE LISTING (136 sequences)

SEQ ID NO: 1 - protein, 472 aa, Homo sapiens
MLYSIFHFGLMMEKKCTLYFLVLLPFFMILVTAELEESPEDSIQLGVTRNKIMTAQYECYQKIMQDPIQQAEGVYCNRTWDGWLCWNDVAAGTESMQLCPDYFQDFDPSEKVTKICDQDGNWFRHPASNRTWTNYTQCNVNTHEKVKTALNLFYLTIIGHGLSIASLLISLGIFFYFKSLSCQRITLHKNLFFSFVCNSVVTIIHLTAVANNQALVATNPVSCKVSQFIHLYLMGCNYFWMLCEGIYLHTLIVVAVFAEKQHLMWYYFLGWGFPLIPACIHAIARSLYYNDNCWISSDTHLLYIIHGPICAALLVNLFFLLNIVRVLITKLKVTHQAESNLYMKAVRATLILVPLLGIEFVLIPWRPEGKIAEEVYDYIMHILMHFQGLLVSTIFCFFNGEVQAILRRNWNQYKIQFGNSFSNSEALRSASYTVSTISDGPGYSHDCPSEHLNGKSIHDIENVLLKPENLYN

SEQ ID NO: 2 - protein, 148 aa, Homo sapiens
MARALCRLPRRGLWLLLAHHLFMTTACQEANYGALLRELCLTQFQVDMEAVGETLWCDWGRTIRSYRELADCTWHMAEKLGCFWPNAEVDRFFLAVHGRYFRSCPISGRAVRDPPGSILYPFIVVPITVTLLVTALVVWQSKRTEGIV

SEQ ID NO: 3 - protein, 116 aa, Homo sapiens
ELEESPEDSIQLGVTRNKIMTAQYECYQKIMQDPIQQAEGVYCNRTWDGWLCWNDVAAGTESMQLCPDYFQDFDPSEKVTKICDQDGNWFRHPASNRTWTNYTQCNVNTHEKVKTA

SEQ ID NO: 4 - protein, 137 aa, Homo sapiens
CQEANYGALLRELCLTQFQVDMEAVGETLWCDWGRTIRSYRELADCCQEANYGALLRELCLTQFQVDMEAVGETLWCDWGRTIRSYRELADCTWHMAEKLGCFWPNAEVDRFFLAVHGRYFRSCPISGRAVRDPPGS

SEQ ID NO: 5 - protein, 17 aa, Artificial Sequence
  Synthetic peptide
DSIQLGVTRNKIMTAQY

SEQ ID NO: 6 - protein, 13 aa, Artificial Sequence
  Synthetic peptide
DVAAGTESMQLCP

SEQ ID NO: 7 - protein, 25 aa, Artificial Sequence
  Synthetic peptide
DGNWFRHPASNRTWTNYTQCNVNTH

SEQ ID NO: 8 - protein, 8 aa, Artificial Sequence
  Synthetic peptide
ECYQKIMQ

SEQ ID NO: 9 - protein, 7 aa, Artificial Sequence
  Synthetic peptide
DGWLCWN

SEQ ID NO: 10 - protein, 12 aa, Artificial Sequence
  Synthetic peptide
RELADCTWHMAE

SEQ ID NO: 11 - protein, 13 aa, Artificial Sequence
  Synthetic peptide
DWGRTIRSYRELA

SEQ ID NO: 12 - protein, 9 aa, Artificial Sequence
  Synthetic peptide
ELCLTQFQV

SEQ ID NO: 13 - protein, 7 aa, Artificial Sequence
  Synthetic peptide
DCTWHMA

SEQ ID NO: 14 - protein, 5 aa, Artificial Sequence
  Synthetic peptide
SFGMH

SEQ ID NO: 15 - protein, 5 aa, Artificial Sequence
  Synthetic peptide
NAWMS

SEQ ID NO: 16 - protein, 5 aa, Artificial Sequence
  Synthetic peptide
SYAMS

SEQ ID NO: 17 - protein, 5 aa, Artificial Sequence
  Synthetic peptide
GYYMH

SEQ ID NO: 18 - protein, 5 aa, Artificial Sequence
  Synthetic peptide
SYGMH

SEQ ID NO: 19 - protein, 5 aa, Artificial Sequence
  Synthetic peptide
DYAMS

SEQ ID NO: 20 - protein, 5 aa, Artificial Sequence
  Synthetic peptide
DYYMY

SEQ ID NO: 21 - protein, 5 aa, Artificial Sequence
  Synthetic peptide
TYSMN

SEQ ID NO: 22 - protein, 5 aa, Artificial Sequence
  Synthetic peptide
SYGMH

SEQ ID NO: 23 - protein, 17 aa, Artificial Sequence
  Synthetic peptide
VISFDGSIKYSVDSVKG

SEQ ID NO: 24 - protein, 19 aa, Artificial Sequence
  Synthetic peptide
RIKSTTDGGTTDYAAPVKG

SEQ ID NO: 25 - protein, 17 aa, Artificial Sequence
  Synthetic peptide
AISGSGGRTYYADSVKG

SEQ ID NO: 26 - protein, 17 aa, Artificial Sequence
  Synthetic peptide
WINPNSGGTNYAQKFQG

SEQ ID NO: 27 - protein, 17 aa, Artificial Sequence
  Synthetic peptide
VISYDGSHESYADSVKG

SEQ ID NO: 28 - protein, 19 aa, Artificial Sequence
  Synthetic peptide
FIRSRAYGGTPEYAASVKG

SEQ ID NO: 29 - protein, 19 aa, Artificial Sequence
  Synthetic peptide
RIKSKTDGGTTDYTAPVKG

SEQ ID NO: 30 - protein, 17 aa, Artificial Sequence
  Synthetic peptide
WISPNSGGTNYAQKFQG

SEQ ID NO: 31 - protein, 19 aa, Artificial Sequence
  Synthetic peptide
RIKSKTDGGTTDYAAPVKG

SEQ ID NO: 32 - protein, 17 aa, Artificial Sequence
  Synthetic peptide
SISSSSSYRYYADSVKG

SEQ ID NO: 33 - protein, 17 aa, Artificial Sequence
  Synthetic peptide
VIWYDGSNKYYADSVKG

SEQ ID NO: 34 - protein, 21 aa, Artificial Sequence
  Synthetic peptide
DRLNYYDSSGYYHYKYYGMAV

SEQ ID NO: 35 - protein, 20 aa, Artificial Sequence
  Synthetic peptide
DRTGYSISWSSYYYYYGMDV

SEQ ID NO: 36 - protein, 21 aa, Artificial Sequence
  Synthetic peptide
DQREVGPYSSGWYDYYYGMDV

SEQ ID NO: 37 - protein, 21 aa, Artificial Sequence
  Synthetic peptide
DQMSIIMLRGVFPPYYYGMDV

SEQ ID NO: 38 - protein, 20 aa, Artificial Sequence
  Synthetic peptide
ERKRVTMSTLYYYFYYGMDV

SEQ ID NO: 39 - protein, 10 aa, Artificial Sequence
  Synthetic peptide
GRGIAARWDY

SEQ ID NO: 40 - protein, 18 aa, Artificial Sequence
  Synthetic peptide
GGYSGYAGLYSHYYGMDV

SEQ ID NO: 41 - protein, 21 aa, Artificial Sequence
  Synthetic peptide
DRLNYYDSSGYYHYKYYGLAV

SEQ ID NO: 42 - protein, 22 aa, Artificial Sequence
  Synthetic peptide
EGVSGSSPYSISWYDYYYGMDV

SEQ ID NO: 43 - protein, 17 aa, Artificial Sequence
  Synthetic peptide
AGGIAAAGLYYYYGMDV

SEQ ID NO: 44 - protein, 13 aa, Artificial Sequence
  Synthetic peptide
SGSSSNIGNNYVS

SEQ ID NO: 45 - protein, 13 aa, Artificial Sequence
  Synthetic peptide
SGSSSNIGSNYVY

SEQ ID NO: 46 - protein, 11 aa, Artificial Sequence
  Synthetic peptide
RASQGIRNDLG

SEQ ID NO: 47 - protein, 11 aa, Artificial Sequence
  Synthetic peptide
QGDSLRSFYAS

SEQ ID NO: 48 - protein, 16 aa, Artificial Sequence
  Synthetic peptide
KSSQSLLHSAGKTYLY

SEQ ID NO: 49 - protein, 16 aa, Artificial Sequence
  Synthetic peptide
RSSQSLLHSFGYNYLD

SEQ ID NO: 50 - protein, 16 aa, Artificial Sequence
  Synthetic peptide
KSSQSLLHSDGKTYLY

SEQ ID NO: 51 - protein, 13 aa, Artificial Sequence
  Synthetic peptide
SGSSSNIGSNTVN

SEQ ID NO: 52 - protein, 16 aa, Artificial Sequence
  Synthetic peptide
KSSQSLLHSDGRNYLY

SEQ ID NO: 53 - protein, 11 aa, Artificial Sequence
  Synthetic peptide
RASQGIRKDLG

SEQ ID NO: 54 - protein, 12 aa, Artificial Sequence
  Synthetic peptide
RASQSVSSGYLT

SEQ ID NO: 55 - protein, 7 aa, Artificial Sequence
  Synthetic peptide
DNNKRPS

SEQ ID NO: 56 - protein, 7 aa, Artificial Sequence
  Synthetic peptide
RSNQRPS

SEQ ID NO: 57 - protein, 7 aa, Artificial Sequence
  Synthetic peptide
AASSLQS

SEQ ID NO: 58 - protein, 7 aa, Artificial Sequence
  Synthetic peptide
GKNNRPS

SEQ ID NO: 59 - protein, 7 aa, Artificial Sequence
  Synthetic peptide
EVSNRFS

SEQ ID NO: 60 - protein, 7 aa, Artificial Sequence
  Synthetic peptide
LGSNRAS

SEQ ID NO: 61 - protein, 7 aa, Artificial Sequence
  Synthetic peptide
RNNQRPS

SEQ ID NO: 62 - protein, 7 aa, Artificial Sequence
  Synthetic peptide
TNNQRPS

SEQ ID NO: 63 - protein, 7 aa, Artificial Sequence
  Synthetic peptide
GASSLQS

SEQ ID NO: 64 - protein, 7 aa, Artificial Sequence
  Synthetic peptide
GASSRAT

SEQ ID NO: 65 - protein, 11 aa, Artificial Sequence
  Synthetic peptide
GTWDSRLSAVV

SEQ ID NO: 66 - protein, 11 aa, Artificial Sequence
  Synthetic peptide
AAWDDSLSGWV

SEQ ID NO: 67 - protein, 9 aa, Artificial Sequence
  Synthetic peptide
LQYNIYPWT

SEQ ID NO: 68 - protein, 11 aa, Artificial Sequence
  Synthetic peptide
NSRDSSVYHLV

SEQ ID NO: 69 - protein, 9 aa, Artificial Sequence
  Synthetic peptide
MQSFPLPLT

SEQ ID NO: 70 - protein, 9 aa, Artificial Sequence
  Synthetic peptide
MQALQTPFT

SEQ ID NO: 71 - protein, 11 aa, Artificial Sequence
  Synthetic peptide
AARDESLNGVV

SEQ ID NO: 72 - protein, 9 aa, Artificial Sequence
  Synthetic peptide
LQYNSFPWT

SEQ ID NO: 73 - protein, 9 aa, Artificial Sequence
  Synthetic peptide
QQYGNSLCR

SEQ ID NO: 74 - protein, 9 aa, Artificial Sequence
  Synthetic peptide
QQYGNSLSR

SEQ ID NO: 75 - protein, 110 aa, Artificial Sequence
  Synthetic peptide
QSVLTQPPSVSEAPGQKVTISCSGSSSNIGNNYVSWYQQLPGTAPKLLIYDNNKRPSGIPDRFSGSKSGTSATLGITGLQTGDEADYYCGTWDSRLSAVVFGGGTKLTVL

SEQ ID NO: 76 - protein, 110 aa, Artificial Sequence
  Synthetic polypeptide
QSVLTQPPSASGTPGQRVTISCSGSSSNIGSNYVYWYQQLPGAAPKLLIFRSNQRPSGVPDRFSGSKSGTSASLAISGLRSEDEADYYCAAWDDSLSGWVFGGGTKLTVL

SEQ ID NO: 77 - protein, 107 aa, Artificial Sequence
  Synthetic polypeptide
DIQMTQSPSSLSASVGDRVTITCRASQGIRNDLGWFQQKPGKAPKRLIYAASSLQSGVPSRFSGSGSGTEFTLTISSLQPEDLATYYCLQYNIYPWTFGQGTKVEIK

SEQ ID NO: 78 - protein, 108 aa, Artificial Sequence
  Synthetic polypeptide
SSELTQDPTVSVALGQTVKITCQGDSLRSFYASWYQQKPGQAPVLVFYGKNNRPSGIPDRFSGSSSGNTASLTITGAQAEDEADYYCNSRDSSVYHLVLGGGTKLTVL

SEQ ID NO: 79 - protein, 112 aa, Artificial Sequence
  Synthetic polypeptide
DIILAQTPLSLSVTPGQPASISCKSSQSLLHSAGKTYLYWYLQKPGQPPQLLIYEVSNRFSGVPDRFSGSGSGTDFTLKISRVEAEDVGIYYCMQSFPLPLTFGGGTKVEIK

SEQ ID NO: 80 - protein, 110 aa, Artificial Sequence
  Synthetic polypeptide
QSVLTQPPSVSAAPGQKVTISCSGSSSNIGNNYVSWYQQLPGTAPKLLIYDNNKRPSGIPDRFSGSKSGTSTTLGITGLQTGDEADYYCGTWDSRLSAVVFGGGTKLTVL

SEQ ID NO: 81 - protein, 112 aa, Artificial Sequence
  Synthetic polypeptide
DIVMTQSPLSLPVTPGEPASISCRSSQSLLHSFGYNYLDWYLQKPGQSPQLLIYLGSNRASGVPDRFSGSGSGTDFTLKISRVEAEDVGVYYCMQALQTPFTFGPGTKVDIK

SEQ ID NO: 82 - protein, 112 aa, Artificial Sequence
  Synthetic polypeptide
DIILTQTPLSLSVTPGQPASISCKSSQSLLHSDGKTYLYWYLQKPGQPPQLLIYEVSNRFSGEPDRFSGSGSGTDFTLKISRVEAEDVGTYYCMQSFPLPLTFGGGTKVEIK

SEQ ID NO: 83 - protein, 110 aa, Artificial Sequence
  Synthetic polypeptide
QSVLTQPPSVSAAPGQKVTISCSGSSSNIGNNYVSWYQQFPGTAPKLLIYDNNKRPSGIPDRFSGSKSGTSATLGITGLQTGDEADYYCGTWDSRLSAVVFGGGTKLTVL

SEQ ID NO: 84 - protein, 110 aa, Artificial Sequence
  Synthetic polypeptide
QSVLTQSPSASGTPGQRVTISCSGSSSNIGSNYVYWYQQLPGAAPKLLILRNNQRPSGVPDRFSGSKSGTSASLTISGLRSEDEADYYCAAWDDSLSGWVFGGGTKLTVL

SEQ ID NO: 85 - protein, 110 aa, Artificial Sequence
  Synthetic polypeptide
QSVLTQPPSASGTPGQRVTISCSGSSSNIGSNTVNWYQQLPGTAPKLLIYTNNQRPSGVPDRFSGSKSGTSASLAISGLQSEDEADFYCAARDESLNGVVFGGGTKLTVL

SEQ ID NO: 86 - protein, 110 aa, Artificial Sequence
  Synthetic polypeptide
QSVLTQPPSASGTPGQRVTISCSGSSSNIGSNYVYWYQQLPGAAPKLLIFRNNQRPSGVPDRFSGSKSGTSASLAISGLRSEDEADYYCAAWDDSLSGWVFGGGTKLTVL

SEQ ID NO: 87 - protein, 112 aa, Artificial Sequence
  Synthetic polypeptide
DITLTQTPLSLSVSPGQPASISCKSSQSLLHSDGRNYLYWYLQKPGQPPQLLIYEVSNRFSGLPDRFSGSGSGTDFTLKISRVEAEDVGIYYCMQSFPLPLTFGGGTKVEIK

SEQ ID NO: 88 - protein, 110 aa, Artificial Sequence
  Synthetic polypeptide
QSVLTQPPSVSAAPGQKVTISCSGSSSNIGNNYVSWYQQLPGTAPKLLIYDNNKRPSGIPDRFSGSKSGTSATLGITGLQTGDEADYYCGTWDSRLSAVVFGGGTKLTVL

SEQ ID NO: 89 - protein, 107 aa, Artificial Sequence
  Synthetic peptide
DIQMTQSPSSLSASVGDRVTITCRASQGIRKDLGWYQQKPGKAPKRLIYGASSLQSGVPSRFSGSGSGTEFTLTISSLQPEDFATYYCLQYNSFPWTFGQGTKVEIK

SEQ ID NO: 90 - protein, 108 aa, Artificial Sequence
  Synthetic polypeptide
EIVLTQSPGTLSLSPGERATLSCRASQSVSSGYLTWYQQKPGQAPRLLIYGASSRATGIPDRFSGSGSGTDFTLTISRLEPEDFAVYYCQQYGNSLCRFGQGTKLEIK

SEQ ID NO: 91 - protein, 108 aa, Artificial Sequence
  Synthetic polypeptide
EIVLTQSPGTLSLSPGERATLSCRASQSVSSGYLTWYQQKPGQAPRLLIYGASSRATGIPDRFSGSGSGTDFTLTISRLEPEDFAVYYCQQYGNSLSRFGQGTKLEIK

SEQ ID NO: 92 - protein, 130 aa, Artificial Sequence [sequence omitted]

SEQ ID NO: 93 - protein, 131 aa, Artificial Sequence
  Synthetic polypeptide
EVQLVESGGGLVKPGGSLRLSCAASGFTFSNAWMSWVRQAPGKGLEWVGRIKSTTDGGTTDYAAPVKGRFTISRDDSKNTLYLQMNSLKTEDTAVYYCTTDRTGYSISWSSYYYYYGMDVWGQGTTVTVSS

SEQ ID NO: 94 - protein, 130 aa, Artificial Sequence
  Synthetic polypeptide
EVQLLESGGGLVQPGESLRLSCAASGFTFSSYAMSWVRQAPGKGLEWVSAISGSGGRTYYADSVKGRFTISRDNSKNTLYLQMNSLRAEDTAVYYCAKDQREVGPYSSGWYDYYYGMDVWGQGTTVTVSS

SEQ ID NO: 95 - protein, 130 aa, Artificial Sequence
  Synthetic polypeptide
QVQLVQSGAEVKKPGASVKVSCKASGYTFTGYYMHWVRQAPGQGLEWMGWINPNSGGTNYAQKFQGRVTMTRDTSISTAYMELSRLRSDDTAVYFCARDQMSIIMLRGVFPPYYYGMDVWGQGTTVTVSS

SEQ ID NO: 96 - protein, 129 aa, Artificial Sequence
  Synthetic polypeptide
QVQLVESGGGVVQPGRSLRLSCAASGFTFSSYGMHWVRQAPGKGLEWVAVISYDGSHESYADSVKGRFTISRDISKNTLYLQMNSLRAEDTAVYFCARERKRVTMSTLYYYFYYGMDVWGQGTTVTVSS

SEQ ID NO: 97 - protein, 121 aa, Artificial Sequence
  Synthetic polypeptide
EVQLVESGGGLVKPGRSLRLSCTASGFTFGDYAMSWFRQAPGKGLEWIGFIRSRAYGGTPEYAASVKGRFTISRDDSKTIAYLQMNSLKTEDTAVYFCARGRGIAARWDYWGQGTLVTVSS

SEQ ID NO: 98 - protein, 131 aa, Artificial Sequence
  Synthetic polypeptide
EVQLVESGGGLVKPGGSLRLSCAASGFTFSNAWMSWVRQAPGKGLEWVGRIKSKTDGGTTDYTAPVKGRFTISRDDSKNTLYLQMNSLKAEDTAVYYCTTDRTGYSISWSSYYYYYGMDVWGQGTTVTVSS

SEQ ID NO: 99 - protein, 127 aa, Artificial Sequence
  Synthetic polypeptide
QVQLVQSGAEVKKPGASVKVSCKASGYTFTDYYMYWVRQAPGQGLEWMGWISPNSGGTNYAQKFQGRVTMTRDTSISTAYMELSRLRSDDTAVYYCVRGGYSGYAGLYSHYYGMDVWGQGTTVTVSS

SEQ ID NO: 100 - protein, 131 aa, Artificial Sequence
  Synthetic polypeptide
EVQLVESGGGLVKPGGSLRLSCAASGFTFGNAWMSWVRQAPGKGLEWVGRIKSKTDGGTTDYAAPVKGRFTISRDDSKNTLYLQMNSLKTEDTAVYFCTTDRTGYSISWSSYYYYYGMDVWGQGTTVTVSS

SEQ ID NO: 101 - protein, 131 aa, Artificial Sequence
  Synthetic polypeptide
EVQLVESGGGLVKPGGSLRLSCAASGFTFGNAWMSWVRQAPGKGLEWVGRIKSKTDGGTTDYAAPVKGRFTISRDDSKNTLYLQMNSLKTEDTAVYYCTTDRTGYSISWSSYYYYYGMDVWGQGTTVTVSS

SEQ ID NO: 102 - protein, 130 aa, Artificial Sequence
  Synthetic polypeptide
QVQLVESGGGVVQPGRSLRLSCAASGFTFSSFGMHWVRQAPGKGLEWVAVISFDGSIKYSVDSVKGRFTISRDNSKNTLFLQMNSLRAEDTAVYYCARDRLNYYDSSGYYHYKYYGLAVWGQGTTVTVSS

SEQ ID NO: 103 - protein, 131 aa, Artificial Sequence
  Synthetic polypeptide
EVQLVESGGGLVKPGGSLRLSCAASGYTFSTYSMNWVRQAPGKGLEWVSSISSSSSYRYYADSVKGRFTISRDNAKNSLYLQMSSLRAEDTAVYYCAREGVSGSSPYSISWYDYYYGMDVWGQGTTVTVSS

SEQ ID NO: 104 - protein, 126 aa, Artificial Sequence
  Synthetic polypeptide
QVQLVESGGGVVQPGRSLRLSCAASGFTFSSYGMHWVRQAPGKGLEWVAVIWYDGSNKYYADSVKGRFIISRDKSKNTLYLQMNSLRAEDTAVYYCARAGGIAAAGLYYYYGMDVWGQGTTVTVSS

SEQ ID NO: 105 - protein, 456 aa, Artificial Sequence
  Synthetic polypeptide
QVQLVESGGGVVQPGRSLRLSCAASGFTFSSFGMHWVRQAPGKGLEWVAVISFDGSIKYSVDSVKGRFTISRDNSKNTLFLQMNSLRAEDTAVYYCARDRLNYYDSSGYYHYKYYGMAVWGQGTTVTVSSASTKGPSVFPLAPCSRSTSESTAALGCLVKDYFPEPVTVSWNSGALTSGVHTFPAVLQSSGLYSLSSVVTVPSSNFGTQTYTCNVDHKPSNTKVDKTVERKCCVECPPCPAPPVAGPSVFLFPPKPKDTLMISRTPEVTCVVVDVSHEDPEVQFNWYVDGVEVHNAKTKPREEQFNSTFRVVSVLTVVHQDWLNGKEYKCKVSNKGLPAPIEKTISKTKGQPREPQVYTLPPSREEMTKNQVSLTCLVKGFYPSDIAVEWESNGQPENNYKTTPPMLDSDGSFFLYSKLTVDKSRWQQGNVFSCSVMHEALHNHYTQKSLSLSPGK

SEQ ID NO: 106 - protein, 457 aa, Artificial Sequence
  Synthetic polypeptide
EVQLVESGGGLVKPGGSLRLSCAASGFTFSNAWMSWVRQAPGKGLEWVGRIKSTTDGGTTDYAAPVKGRFTISRDDSKNTLYLQMNSLKTEDTAVYYCTTDRTGYSISWSSYYYYYGMDVWGQGTTVTVSSASTKGPSVFPLAPCSRSTSESTAALGCLVKDYFPEPVTVSWNSGALTSGVHTFPAVLQSSGLYSLSSVVTVPSSNFGTQTYTCNVDHKPSNTKVDKTVERKCCVECPPCPAPPVAGPSVFLFPPKPKDTLMISRTPEVTCVVVDVSHEDPEVQFNWYVDGVEVHNAKTKPREEQFNSTFRVVSVLTVVHQDWLNGKEYKCKVSNKGLPAPIEKTISKTKGQPREPQVYTLPPSREEMTKNQVSLTCLVKGFYPSDIAVEWESNGQPENNYKTTPPMLDSDGSFFLYSKLTVDKSRWQQGNVFSCSVMHEALHNHYTQKSLSLSPGK

SEQ ID NO: 107 - protein, 456 aa, Artificial Sequence
  Synthetic polypeptide
EVQLLESGGGLVQPGESLRLSCAASGFTFSSYAMSWVRQAPGKGLEWVSAISGSGGRTYYADSVKGRFTISRDNSKNTLYLQMNSLRAEDTAVYYCAKDQREVGPYSSGWYDYYYGMDVWGQGTTVTVSSASTKGPSVFPLAPCSRSTSESTAALGCLVKDYFPEPVTVSWNSGALTSGVHTFPAVLQSSGLYSLSSVVTVPSSNFGTQTYTCNVDHKPSNTKVDKTVERKCCVECPPCPAPPVAGPSVFLFPPKPKDTLMISRTPEVTCVVVDVSHEDPEVQFNWYVDGVEVHNAKTKPREEQFNSTFRVVSVLTVVHQDWLNGKEYKCKVSNKGLPAPIEKTISKTKGQPREPQVYTLPPSREEMTKNQVSLTCLVKGFYPSDIAVEWESNGQPENNYKTTPPMLDSDGSFFLYSKLTVDKSRWQQGNVFSCSVMHEALHNHYTQKSLSLSPGK

SEQ ID NO: 108 - protein, 456 aa, Artificial Sequence
  Synthetic polypeptide
QVQLVQSGAEVKKPGASVKVSCKASGYTFTGYYMHWVRQAPGQGLEWMGWINPNSGGTNYAQKFQGRVTMTRDTSISTAYMELSRLRSDDTAVYFCARDQMSIIMLRGVFPPYYYGMDVWGQGTTVTVSSASTKGPSVFPLAPCSRSTSESTAALGCLVKDYFPEPVTVSWNSGALTSGVHTFPAVLQSSGLYSLSSVVTVPSSNFGTQTYTCNVDHKPSNTKVDKTVERKCCVECPPCPAPPVAGPSVFLFPPKPKDTLMISRTPEVTCVVVDVSHEDPEVQFNWYVDGVEVHNAKTKPREEQFNSTFRVVSVLTVVHQDWLNGKEYKCKVSNKGLPAPIEKTISKTKGQPREPQVYTLPPSREEMTKNQVSLTCLVKGFYPSDIAVEWESNGQPENNYKTTPPMLDSDGSFFLYSKLTVDKSRWQQGNVFSCSVMHEALHNHYTQKSLSLSPGK

SEQ ID NO: 109 - protein, 455 aa, Artificial Sequence
  Synthetic polypeptide
QVQLVESGGGVVQPGRSLRLSCAASGFTFSSYGMHWVRQAPGKGLEWVAVISYDGSHESYADSVKGRFTISRDISKNTLYLQMNSLRAEDTAVYFCARERKRVTMSTLYYYFYYGMDVWGQGTTVTVSSASTKGPSVFPLAPCSRSTSESTAALGCLVKDYFPEPVTVSWNSGALTSGVHTFPAVLQSSGLYSLSSVVTVPSSNFGTQTYTCNVDHKPSNTKVDKTVERKCCVECPPCPAPPVAGPSVFLFPPKPKDTLMISRTPEVTCVVVDVSHEDPEVQFNWYVDGVEVHNAKTKPREEQFNSTFRVVSVLTVVHQDWLNGKEYKCKVSNKGLPAPIEKTISKTKGQPREPQVYTLPPSREEMTKNQVSLTCLVKGFYPSDIAVEWESNGQPENNYKTTPPMLDSDGSFFLYSKLTVDKSRWQQGNVFSCSVMHEALHNHYTQKSLSLSPGK

SEQ ID NO: 110 - protein, 447 aa, Artificial Sequence
  Synthetic polypeptide
EVQLVESGGGLVKPGRSLRLSCTASGFTFGDYAMSWFRQAPGKGLEWIGFIRSRAYGGTPEYAASVKGRFTISRDDSKTIAYLQMNSLKTEDTAVYFCARGRGIAARWDYWGQGTLVTVSSASTKGPSVFPLAPCSRSTSESTAALGCLVKDYFPEPVTVSWNSGALTSGVHTFPAVLQSSGLYSLSSVVTVPSSNFGTQTYTCNVDHKPSNTKVDKTVERKCCVECPPCPAPPVAGPSVFLFPPKPKDTLMISRTPEVTCVVVDVSHEDPEVQFNWYVDGVEVHNAKTKPREEQFNSTFRVVSVLTVVHQDWLNGKEYKCKVSNKGLPAPIEKTISKTKGQPREPQVYTLPPSREEMTKNQVSLTCLVKGFYPSDIAVEWESNGQPENNYKTTPPMLDSDGSFFLYSKLTVDKSRWQQGNVFSCSVMHEALHNHYTQKSLSLSPGK

SEQ ID NO: 111 - protein, 457 aa, Artificial Sequence
  Synthetic polypeptide
EVQLVESGGGLVKPGGSLRLSCAASGFTFSNAWMSWVRQAPGKGLEWVGRIKSKTDGGTTDYTAPVKGRFTISRDDSKNTLYLQMNSLKAEDTAVYYCTTDRTGYSISWSSYYYYYGMDVWGQGTTVTVSSASTKGPSVFPLAPCSRSTSESTAALGCLVKDYFPEPVTVSWNSGALTSGVHTFPAVLQSSGLYSLSSVVTVPSSNFGTQTYTCNVDHKPSNTKVDKTVERKCCVECPPCPAPPVAGPSVFLFPPKPKDTLMISRTPEVTCVVVDVSHEDPEVQFNWYVDGVEVHNAKTKPREEQFNSTFRVVSVLTVVHQDWLNGKEYKCKVSNKGLPAPIEKTISKTKGQPREPQVYTLPPSREEMTKNQVSLTCLVKGFYPSDIAVEWESNGQPENNYKTTPPMLDSDGSFFLYSKLTVDKSRWQQGNVFSCSVMHEALHNHYTQKSLSLSPGK

SEQ ID NO: 112 - protein, 453 aa, Artificial Sequence
  Synthetic polypeptide
QVQLVQSGAEVKKPGASVKVSCKASGYTFTDYYMYWVRQAPGQGLEWMGWISPNSGGTNYAQKFQGRVTMTRDTSISTAYMELSRLRSDDTAVYYCVRGGYSGYAGLYSHYYGMDVWGQGTTVTVSSASTKGPSVFPLAPCSRSTSESTAALGCLVKDYFPEPVTVSWNSGALTSGVHTFPAVLQSSGLYSLSSVVTVPSSNFGTQTYTCNVDHKPSNTKVDKTVERKCCVECPPCPAPPVAGPSVFLFPPKPKDTLMISRTPEVTCVVVDVSHEDPEVQFNWYVDGVEVHNAKTKPREEQFNSTFRVVSVLTVVHQDWLNGKEYKCKVSNKGLPAPIEKTISKTKGQPREPQVYTLPPSREEMTKNQVSLTCLVKGFYPSDIAVEWESNGQPENNYKTTPPMLDSDGSFFLYSKLTVDKSRWQQGNVFSCSVMHEALHNHYTQKSLSLSPGK

SEQ ID NO: 113 - protein, 457 aa, Artificial Sequence
  Synthetic polypeptide
EVQLVESGGGLVKPGGSLRLSCAASGFTFGNAWMSWVRQAPGKGLEWVGRIKSKTDGGTTDYAAPVKGRFTISRDDSKNTLYLQMNSLKTEDTAVYFCTTDRTGYSISWSSYYYYYGMDVWGQGTTVTVSSASTKGPSVFPLAPCSRSTSESTAALGCLVKDYFPEPVTVSWNSGALTSGVHTFPAVLQSSGLYSLSSVVTVPSSNFGTQTYTCNVDHKPSNTKVDKTVERKCCVECPPCPAPPVAGPSVFLFPPKPKDTLMISRTPEVTCVVVDVSHEDPEVQFNWYVDGVEVHNAKTKPREEQFNSTFRVVSVLTVVHQDWLNGKEYKCKVSNKGLPAPIEKTISKTKGQPREPQVYTLPPSREEMTKNQVSLTCLVKGFYPSDIAVEWESNGQPENNYKTTPPMLDSDGSFFLYSKLTVDKSRWQQGNVFSCSVMHEALHNHYTQKSLSLSPGK

SEQ ID NO: 114 - protein, 457 aa, Artificial Sequence
  Synthetic polypeptide
EVQLVESGGGLVKPGGSLRLSCAASGFTFGNAWMSWVRQAPGKGLEWVGRIKSKTDGGTTDYAAPVKGRFTISRDDSKNTLYLQMNSLKTEDTAVYYCTTDRTGYSISWSSYYYYYGMDVWGQGTTVTVSSASTKGPSVFPLAPCSRSTSESTAALGCLVKDYFPEPVTVSWNSGALTSGVHTFPAVLQSSGLYSLSSVVTVPSSNFGTQTYTCNVDHKPSNTKVDKTVERKCCVECPPCPAPPVAGPSVFLFPPKPKDTLMISRTPEVTCVVVDVSHEDPEVQFNWYVDGVEVHNAKTKPREEQFNSTFRVVSVLTVVHQDWLNGKEYKCKVSNKGLPAPIEKTISKTKGQPREPQVYTLPPSREEMTKNQVSLTCLVKGFYPSDIAVEWESNGQPENNYKTTPPMLDSDGSFFLYSKLTVDKSRWQQGNVFSCSVMHEALHNHYTQKSLSLSPGK

SEQ ID NO: 115 - protein, 456 aa, Artificial Sequence
  Synthetic polypeptide
QVQLVESGGGVVQPGRSLRLSCAASGFTFSSFGMHWVRQAPGKGLEWVAVISFDGSIKYSVDSVKGRFTISRDNSKNTLFLQMNSLRAEDTAVYYCARDRLNYYDSSGYYHYKYYGLAVWGQGTTVTVSSASTKGPSVFPLAPCSRSTSESTAALGCLVKDYFPEPVTVSWNSGALTSGVHTFPAVLQSSGLYSLSSVVTVPSSNFGTQTYTCNVDHKPSNTKVDKTVERKCCVECPPCPAPPVAGPSVFLFPPKPKDTLMISRTPEVTCVVVDVSHEDPEVQFNWYVDGVEVHNAKTKPREEQFNSTFRVVSVLTVVHQDWLNGKEYKCKVSNKGLPAPIEKTISKTKGQPREPQVYTLPPSREEMTKNQVSLTCLVKGFYPSDIAVEWESNGQPENNYKTTPPMLDSDGSFFLYSKLTVDKSRWQQGNVFSCSVMHEALHNHYTQKSLSLSPGK

SEQ ID NO: 116 - protein, 457 aa, Artificial Sequence
  Synthetic polypeptide
EVQLVESGGGLVKPGGSLRLSCAASGYTFSTYSMNWVRQAPGKGLEWVSSISSSSSYRYYADSVKGRFTISRDNAKNSLYLQMSSLRAEDTAVYYCAREGVSGSSPYSISWYDYYYGMDVWGQGTTVTVSSASTKGPSVFPLAPCSRSTSESTAALGCLVKDYFPEPVTVSWNSGALTSGVHTFPAVLQSSGLYSLSSVVTVPSSNFGTQTYTCNVDHKPSNTKVDKTVERKCCVECPPCPAPPVAGPSVFLFPPKPKDTLMISRTPEVTCVVVDVSHEDPEVQFNWYVDGVEVHNAKTKPREEQFNSTFRVVSVLTVVHQDWLNGKEYKCKVSNKGLPAPIEKTISKTKGQPREPQVYTLPPSREEMTKNQVSLTCLVKGFYPSDIAVEWESNGQPENNYKTTPPMLDSDGSFFLYSKLTVDKSRWQQGNVFSCSVMHEALHNHYTQKSLSLSPGK

SEQ ID NO: 117 - protein, 452 aa, Artificial Sequence
  Synthetic polypeptide
QVQLVESGGGVVQPGRSLRLSCAASGFTFSSYGMHWVRQAPGKGLEWVAVIWYDGSNKYYADSVKGRFIISRDKSKNTLYLQMNSLRAEDTAVYYCARAGGIAAAGLYYYYGMDVWGQGTTVTVSSASTKGPSVFPLAPCSRSTSESTAALGCLVKDYFPEPVTVSWNSGALTSGVHTFPAVLQSSGLYSLSSVVTVPSSNFGTQTYTCNVDHKPSNTKVDKTVERKCCVECPPCPAPPVAGPSVFLFPPKPKDTLMISRTPEVTCVVVDVSHEDPEVQFNWYVDGVEVHNAKTKPREEQFNSTFRVVSVLTVVHQDWLNGKEYKCKVSNKGLPAPIEKTISKTKGQPREPQVYTLPPSREEMTKNQVSLTCLVKGFYPSDIAVEWESNGQPENNYKTTPPMLDSDGSFFLYSKLTVDKSRWQQGNVFSCSVMHEALHNHYTQKSLSLSPGK

SEQ ID NO: 118 - protein, 216 aa, Artificial Sequence
  Synthetic polypeptide
QSVLTQPPSVSEAPGQKVTISCSGSSSNIGNNYVSWYQQLPGTAPKLLIYDNNKRPSGIPDRFSGSKSGTSATLGITGLQTGDEADYYCGTWDSRLSAVVFGGGTKLTVLGQPKANPTVTLFPPSSEELQANKATLVCLISDFYPGAVTVAWKADGSPVKAGVETTKPSKQSNNKYAASSYLSLTPEQWKSHRSYSCQVTHEGSTVEKTVAPTECS

SEQ ID NO: 119 - protein, 216 aa, Artificial Sequence
  Synthetic polypeptide
QSVLTQPPSASGTPGQRVTISCSGSSSNIGSNYVYWYQQLPGAAPKLLIFRSNQRPSGVPDRFSGSKSGTSASLAISGLRSEDEADYYCAAWDDSLSGWVFGGGTKLTVLGQPKANPTVTLFPPSSEELQANKATLVCLISDFYPGAVTVAWKADGSPVKAGVETTKPSKQSNNKYAASSYLSLTPEQWKSHRSYSCQVTHEGSTVEKTVAPTECS

SEQ ID NO: 120 - protein, 214 aa, Artificial Sequence
  Synthetic polypeptide
DIQMTQSPSSLSASVGDRVTITCRASQGIRNDLGWFQQKPGKAPKRLIYAASSLQSGVPSRFSGSGSGTEFTLTISSLQPEDLATYYCLQYNIYPWTFGQGTKVEIKRTVAAPSVFIFPPSDEQLKSGTASVVCLLNNFYPREAKVQWKVDNALQSGNSQESVTEQDSKDSTYSLSSTLTLSKADYEKHKVYACEVTHQGLSSPVTKSFNRGEC

SEQ ID NO: 121 - protein, 214 aa, Artificial Sequence
  Synthetic polypeptide
SSELTQDPTVSVALGQTVKITCQGDSLRSFYASWYQQKPGQAPVLVFYGKNNRPSGIPDRFSGSSSGNTASLTITGAQAEDEADYYCNSRDSSVYHLVLGGGTKLTVLGQPKANPTVTLFPPSSEELQANKATLVCLISDFYPGAVTVAWKADGSPVKAGVETTKPSKQSNNKYAASSYLSLTPEQWKSHRSYSCQVTHEGSTVEKTVAPTECS

SEQ ID NO: 122 - protein, 219 aa, Artificial Sequence
  Synthetic polypeptide
DIILAQTPLSLSVTPGQPASISCKSSQSLLHSAGKTYLYWYLQKPGQPPQLLIYEVSNRFSGVPDRFSGSGSGTDFTLKISRVEAEDVGIYYCMQSFPLPLTFGGGTKVEIKRTVAAPSVFIFPPSDEQLKSGTASVVCLLNNFYPREAKVQWKVDNALQSGNSQESVTEQDSKDSTYSLSSTLTLSKADYEKHKVYACEVTHQGLSSPVTKSFNRGEC

SEQ ID NO: 123 - protein, 216 aa, Artificial Sequence
  Synthetic polypeptide
QSVLTQPPSVSAAPGQKVTISCSGSSSNIGNNYVSWYQQLPGTAPKLLIYDNNKRPSGIPDRFSGSKSGTSTTLGITGLQTGDEADYYCGTWDSRLSAVVFGGGTKLTVLGQPKANPTVTLFPPSSEELQANKATLVCLISDFYPGAVTVAWKADGSPVKAGVETTKPSKQSNNKYAASSYLSLTPEQWKSHRSYSCQVTHEGSTVEKTVAPTECS

SEQ ID NO: 124 - protein, 219 aa, Artificial Sequence
  Synthetic polypeptide
DIVMTQSPLSLPVTPGEPASISCRSSQSLLHSFGYNYLDWYLQKPGQSPQLLIYLGSNRASGVPDRFSGSGSGTDFTLKISRVEAEDVGVYYCMQALQTPFTFGPGTKVDIKRTVAAPSVFIFPPSDEQLKSGTASVVCLLNNFYPREAKVQWKVDNALQSGNSQESVTEQDSKDSTYSLSSTLTLSKADYEKHKVYACEVTHQGLSSPVTKSFNRGEC

SEQ ID NO: 125 - protein, 219 aa, Artificial Sequence
  Synthetic polypeptide
DIILTQTPLSLSVTPGQPASISCKSSQSLLHSDGKTYLYWYLQKPGQPPQLLIYEVSNRFSGEPDRFSGSGSGTDFTLKISRVEAEDVGTYYCMQSFPLPLTFGGGTKVEIKRTVAAPSVFIFPPSDEQLKSGTASVVCLLNNFYPREAKVQWKVDNALQSGNSQESVTEQDSKDSTYSLSSTLTLSKADYEKHKVYACEVTHQGLSSPVTKSFNRGEC

SEQ ID NO: 126 - protein, 216 aa, Artificial Sequence
  Synthetic polypeptide
QSVLTQPPSVSAAPGQKVTISCSGSSSNIGNNYVSWYQQFPGTAPKLLIYDNNKRPSGIPDRFSGSKSGTSATLGITGLQTGDEADYYCGTWDSRLSAVVFGGGTKLTVLGQPKANPTVTLFPPSSEELQANKATLVCLISDFYPGAVTVAWKADGSPVKAGVETTKPSKQSNNKYAASSYLSLTPEQWKSHRSYSCQVTHEGSTVEKTVAPTECS

SEQ ID NO: 127 - protein, 216 aa, Artificial Sequence
  Synthetic polypeptide
QSVLTQSPSASGTPGQRVTISCSGSSSNIGSNYVYWYQQLPGAAPKLLILRNNQRPSGVPDRFSGSKSGTSASLTISGLRSEDEADYYCAAWDDSLSGWVFGGGTKLTVLGQPKANPTVTLFPPSSEELQANKATLVCLISDFYPGAVTVAWKADGSPVKAGVETTKPSKQSNNKYAASSYLSLTPEQWKSHRSYSCQVTHEGSTVEKTVAPTECS

SEQ ID NO: 128 - protein, 216 aa, Artificial Sequence
  Synthetic polypeptide
QSVLTQPPSASGTPGQRVTISCSGSSSNIGSNTVNWYQQLPGTAPKLLIYTNNQRPSGVPDRFSGSKSGTSASLAISGLQSEDEADFYCAARDESLNGVVFGGGTKLTVLGQPKANPTVTLFPPSSEELQANKATLVCLISDFYPGAVTVAWKADGSPVKAGVETTKPSKQSNNKYAASSYLSLTPEQWKSHRSYSCQVTHEGSTVEKTVAPTECS

SEQ ID NO: 129 - protein, 216 aa, Artificial Sequence
  Synthetic polypeptide
QSVLTQPPSASGTPGQRVTISCSGSSSNIGSNYVYWYQQLPGAAPKLLIFRNNQRPSGVPDRFSGSKSGTSASLAISGLRSEDEADYYCAAWDDSLSGWVFGGGTKLTVLGQPKANPTVTLFPPSSEELQANKATLVCLISDFYPGAVTVAWKADGSPVKAGVETTKPSKQSNNKYAASSYLSLTPEQWKSHRSYSCQVTHEGSTVEKTVAPTECS

SEQ ID NO: 130 - protein, 219 aa, Artificial Sequence
  Synthetic polypeptide
DITLTQTPLSLSVSPGQPASISCKSSQSLLHSDGRNYLYWYLQKPGQPPQLLIYEVSNRFSGLPDRFSGSGSGTDFTLKISRVEAEDVGIYYCMQSFPLPLTFGGGTKVEIKRTVAAPSVFIFPPSDEQLKSGTASVVCLLNNFYPREAKVQWKVDNALQSGNSQESVTEQDSKDSTYSLSSTLTLSKADYEKHKVYACEVTHQGLSSPVTKSFNRGEC

SEQ ID NO: 131 - protein, 216 aa, Artificial Sequence
  Synthetic polypeptide
QSVLTQPPSVSAAPGQKVTISCSGSSSNIGNNYVSWYQQLPGTAPKLLIYDNNKRPSGIPDRFSGSKSGTSATLGITGLQTGDEADYYCGTWDSRLSAVVFGGGTKLTVLGQPKANPTVTLFPPSSEELQANKATLVCLISDFYPGAVTVAWKADGSPVKAGVETTKPSKQSNNKYAASSYLSLTPEQWKSHRSYSCQVTHEGSTVEKTVAPTECS

SEQ ID NO: 132 - protein, 214 aa, Artificial Sequence
  Synthetic polypeptide
DIQMTQSPSSLSASVGDRVTITCRASQGIRKDLGWYQQKPGKAPKRLIYGASSLQSGVPSRFSGSGSGTEFTLTISSLQPEDFATYYCLQYNSFPWTFGQGTKVEIKRTVAAPSVFIFPPSDEQLKSGTASVVCLLNNFYPREAKVQWKVDNALQSGNSQESVTEQDSKDSTYSLSSTLTLSKADYEKHKVYACEVTHQGLSSPVTKSFNRGEC

SEQ ID NO: 133 - protein, 215 aa, Artificial Sequence
  Synthetic polypeptide
EIVLTQSPGTLSLSPGERATLSCRASQSVSSGYLTWYQQKPGQAPRLLIYGASSRATGIPDRFSGSGSGTDFTLTISRLEPEDFAVYYCQQYGNSLCRFGQGTKLEIKRTVAAPSVFIFPPSDEQLKSGTASVVCLLNNFYPREAKVQWKVDNALQSGNSQESVTEQDSKDSTYSLSSTLTLSKADYEKHKVYACEVTHQGLSSPVTKSFNRGEC

SEQ ID NO: 134 - protein, 215 aa, Artificial Sequence
  Synthetic polypeptide
EIVLTQSPGTLSLSPGERATLSCRASQSVSSGYLTWYQQKPGQAPRLLIYGASSRATGIPDRFSGSGSGTDFTLTISRLEPEDFAVYYCQQYGNSLSRFGQGTKLEIKRTVAAPSVFIFPPSDEQLKSGTASVVCLLNNFYPREAKVQWKVDNALQSGNSQESVTEQDSKDSTYSLSSTLTLSKADYEKHKVYACEVTHQGLSSPVTKSFNRGEC

SEQ ID NO: 135 - protein, 22 aa, Artificial Sequence
  Synthetic peptide
MDMRVPAQLLGLLLLWLRGARC

SEQ ID NO: 136 - protein, 20 aa, Artificial Sequence
  Synthetic peptide
METPAQLLFLLLLWLPDTTG